European Patent Application EP 4 151 785 A1, published March 22, 2023. Title: FIBRONECTIN TYPE III REPEAT BASED PROTEIN SCAFFOLDS WITH ALTERNATIVE BINDING SURFACES. Applicant: Janssen Biotech, Inc. The sequence listing filed with the application follows.

SEQUENCE LISTING (101 sequences)

SEQ ID NO: 1 - protein, 87 aa, homo sapiens
SPPKDLVVTEVTEETVNLAWDNEMRVTEYLVVYTPTHEGGLEMQFRVPGDQTSTIIQELEPGVEYFIRVFAILENKKSIPVSARVAT

SEQ ID NO: 2 - protein, 95 aa, homo sapiens
TYLPAPEGLKFKSIKETSVEVEWDPLDIAFETWEIIFRNMNKEDEGEITKSLRRPETSYRQTGLAPGQEYEISLHIVKNNTRGPGLKRVTTTRLD

SEQ ID NO: 3 - protein, 88 aa, homo sapiens
DAPSQIEVKDVTDTTALITWFKPLAEIDGIELTYGIKDVPGDRTTIDLTEDENQYSIGNLKPDTEYEVSLISRRGDMSSNPAKETFTT

SEQ ID NO: 4 - protein, 100 aa, homo sapiens
TGLDAPRNLRRVSQTDNSITLEWRNGKAAIDSYRIKYAPISGGDHAEVDVPKSQQATTKTTLTGLRPGTEYGIGVSAVKEDKESNPATINAATELDTPKD

SEQ ID NO: 5 - protein, 88 aa, homo sapiens
DTPKDLQVSETAETSLTLLWKTPLAKFDRYRLNYSLPTGQWVGVQLPRNTTSYVLRGLEPGQEYNVLLTAEKGRHKSKPAKSKPARVK

SEQ ID NO: 6 - protein, 92 aa, homo sapiens
QAPELENLTVTEVGWDGLRLNWTAADQAYEHFIIQVQEANKVEAARNLTVPGSLRAVDIPGLKAATPYTVSIYGVIQGYRTPVLSAEASTGE

SEQ ID NO: 7 - protein, 91 aa, homo sapiens
ETPNLGEVVVAEVGWDALKLNWTAPEGAYEYFFIQVQEADTVEAAQNLTVPGGLRSTDLPGLKAATHYTITIRGVTQDFSTTPLSVEVLTE

SEQ ID NO: 8 - protein, 91 aa, homo sapiens
EVPDMGNLTVTEVSWDALRLNWTTPDGTYDQFTIQVQEADQVEEAHNLTVPGSLRSMEIPGLRAGTPYTVTLHGEVRGHSTRPLAVEVVTE

SEQ ID NO: 9 - protein, 95 aa, homo sapiens
DLPQLGDLAVSEVGWDGLRLNWTAADNAYEHFVIQVQEVNKVEAAQNLTLPGSLRAVDIPGLEAATPYRVSIYGVIRGYRTPVLSAEASTAKEPE

SEQ ID NO: 10 - protein, 91 aa, homo sapiens
KEPEIGNLNVSDITPESFNLSWMATDGIFETFTIEIIDSNRLLETVEYNISGAERTAHISGLPPSTDFIVYLSGLAPSIRTKTISATATTE

SEQ ID NO: 11 - protein, 91 aa, homo sapiens
ALPLLENLTISDINPYGFTVSWMASENAFDSFLVTVVDSGKLLDPQEFTLSGTQRKLELRGLITGIGYEVMVSGFTQGHQTKPLRAEIVTE

SEQ ID NO: 12 - protein, 92 aa, homosapiens
AEPEVDNLLVSDATPDGFRLSWTADEGVFDNFVLKIRDTKKQSEPLEITLLAPERTRDLTGLREATEYEIELYGISKGRRSQTVSAIATTAM

SEQ ID NO: 13 - protein, 89 aa, homo sapiens
GSPKEVIFSDITENSATVSWRAPTAQVESFRITYVPITGGTPSMVTVDGTKTQTRLVKLIPGVEYLVSIIAMKGFEESEPVSGSFTTAL

SEQ ID NO: 14 - protein, 88 aa, homo sapiens
DGPSGLVTANITDSEALARWQPAIATVDSYVISYTGEKVPEITRTVSGNTVEYALTDLEPATEYTLRIFAEKGPQKSSTITAKFTTDL

SEQ ID NO: 15 - protein, 89 aa, homosapiens
DSPRDLTATEVQSETALLTWRPPRASVTGYLLVYESVDGTVKEVIVGPDTTSYSLADLSPSTHYTAKIQALNGPLRSNMIQTIFTTIGL

SEQ ID NO: 16 - protein, 89 aa, synthetic construct
  REGION 1..89: note = Consensus FN3 sequence based on tenascin C FN3 domains
LPAPKNLVVSEVTEDSLRLSWTAPDAAFDSFLIQYQESEKVGEAINLTVPGSERSYDLTGLKPGTEYTVSIYGVKGGHRSNPLSAEFTT

SEQ ID NO: 17 - protein, 89 aa, synthetic construct
  REGION 1..89: note = Consensus FN3 sequence based on tenascin C FN3 domains withadditional mutations improving stability
LPAPKNLVVSEVTEDSLRLSWTAPDAAFDSFLIQYQESEKVGEAIVLTVPGSERSYDLTGLKPGTEYTVSIYGVKGGHRSNPLSAEFTT

SEQ ID NO: 18 - protein, 89 aa, synthetic construct
  REGION 1..89: note = Consensus FN3 sequence based on tenascin C FN3 domains withadditional mutations improving stability
LPAPKNLVVSEVTPDSLRLSWTAPDAAFDSFLIQYQESEKVGEAINLTVPGSERSYDLTGLKPGTEYTVSIYGVKGGHRSNPLSAEFTT

SEQ ID NO: 19 - protein, 89 aa, synthetic construct
  REGION 1..89: note = Consensus FN3 sequence based on tenascin C FN3 domains withadditional mutations improving stability
LPAPKNLVVSNVTEDSLRLSWTAPDAAFDSFLIQYQESEKVGEAINLTVPGSERSYDLTGLKPGTEYTVSIYGVKGGHRSNPLSAEFTT

SEQ ID NO: 20 - protein, 89 aa, synthetic construct
  REGION 1..89: note = Consensus FN3 sequence based on tenascin C FN3 domains withadditional mutations improving stability
LPAPKNLVVSEVTEDSLRLSWTAPDAAFDSFLIQYQPSEKVGEAINLTVPGSERSYDLTGLKPGTEYTVSIYGVKGGHRSNPLSAEFTT

SEQ ID NO: 21 - protein, 89 aa, synthetic construct
  REGION 1..89: note = Consensus FN3 sequence based on tenascin C FN3 domains withadditional mutations improving stability
LPAPKNLVVSEVTEDSLRLSWTAPDAAFDSFLIQYQESEKVGEAINLTVPGSERSYDLTGLKPGTEYTVSIYYVKGGHRSNPLSAEFTT

SEQ ID NO: 22 - protein, 89 aa, synthetic construct
  REGION 1..89: note = Consensus FN3 sequence based on tenascin C FN3 domains withadditional mutations improving stability
LPAPKNLVVSEVTEDSLRLSWTAPDAAFDSFLIQYQESEKVGEAINLTVPGSERSYDLTGLKPGTEYTVSIYGVKGGHRSNPLSAIFTT

SEQ ID NO: 23 - protein, 89 aa, synthetic construct
  REGION 1..89: note = Consensus FN3 sequence based on tenascin C FN3 domains withadditional mutations improving stability
LPAPKNLVVSEVTEDSLRLSWTAPDAAFDSFLIQYQESEKVGEAIVLTVPGSERSYDLTGLKPGTEYTVSIYGVKGGHRSNPLSAIFTT

SEQ ID NO: 24 - protein, 89 aa, synthetic construct
  REGION 1..89: note = Consensus FN3 sequence based on tenascin C FN3 domains withadditional mutations improving stability
LPAPKNLVVSEVTPDSLRLSWTAPDAAFDSFLIQYQESEKVGEAIVLTVPGSERSYDLTGLKPGTEYTVSIYGVKGGHRSNPLSAIFTT

SEQ ID NO: 25 - protein, 89 aa, synthetic construct
  REGION 1..89: note = Consensus FN3 sequence based on tenascin C FN3 domains withadditional mutations improving stability
LPAPKNLVVSEVTEDSARLSWTAPDAAFDSFLIQYQESEKVGEAIVLTVPGSERSYDLTGLKPGTEYTVSIYGVKGGHRSNPLSAIFTT

SEQ ID NO: 26 - protein, 89 aa, synthetic construct
  REGION 1..89: note = Consensus FN3 sequence based on tenascin C FN3 domains withadditional mutations improving stability
LPAPKNLVVSEVTEDSARLSWTAPDAAFDSFLIQYQESEKVGEAINLTVPGSERSYDLTGLKPGTEYTVSIYGVKGGHRSNPLSAEFTT

SEQ ID NO: 27 - protein, 89 aa, synthetic construct
  REGION 1..89: note = Consensus FN3 sequence based on tenascin C FN3 domains withadditional mutations improving stability
LPAPKNLVVSRVTEDSARLSWTAPDAAFDSFLIQYQESEKVGEAIVLTVPGSERSYDLTGLKPGTEYTVSIYGVKGGHRSNPLSAIFTT

SEQ ID NO: 28 - protein, 89 aa, synthetic construct
  REGION 1..89: note = TCL14 library based on tencon27 scaffold with randomizedC-CD-F-FG surface
  SITE 32: note = misc_feature - Xaa can be any naturally occurring amino acid
  SITE 34: note = misc_feature - Xaa can be any naturally occurring amino acid
  SITE 36: note = misc_feature - Xaa can be any naturally occurring amino acid
  REGION 38..41: note = misc_feature - Xaa can be any naturally occurring amino acid
  SITE 68: note = misc_feature - Xaa can be any naturally occurring amino acid
  SITE 70: note = misc_feature - Xaa can be any naturally occurring amino acid
  SITE 72: note = misc_feature - Xaa can be any naturally occurring amino acid
  REGION 78..79: note = misc_feature - Xaa can be any naturally occurring amino acid
  SITE 81: note = misc_feature - Xaa can be any naturally occurring amino acid
LPAPKNLVVSRVTEDSARLSWTAPDAAFDSFXIXYXEXXXXGEAIVLTVPGSERSYDLTGLKPGTEYXVXIXGVKGGXXSXPLSAIFTT

SEQ ID NO: 29 - protein, 12 aa, synthetic construct
  REGION 1..12: note = Tencon27 scaffold A strand sequence
LPAPKNLVVSRV

SEQ ID NO: 30 - protein, 4 aa, synthetic construct
  REGION 1..4: note = Tencon27 scaffold AB loop
TEDS

SEQ ID NO: 31 - protein, 5 aa, synthetic construct
  REGION 1..5: note = Tencon27 scaffold B strand
ARLSW

SEQ ID NO: 32 - protein, 7 aa, synthetic construct
  REGION 1..7: note = Tencon27 scaffold BC loop
TAPDAAF

SEQ ID NO: 33 - protein, 9 aa, synthetic construct
  REGION 1..9: note = Tencon27 scaffold C strand
DSFLIQYQE

SEQ ID NO: 34 - protein, 6 aa, synthetic construct
  REGION 1..6: note = Tencon27 scaffold CD loop
SEKVGE

SEQ ID NO: 35 - protein, 7 aa, synthetic construct
  REGION 1..7: note = Tencon27 scaffold D strand
AIVLTVP

SEQ ID NO: 36 - protein, 4 aa, synthetic construct
  REGION 1..4: note = Tencon27 scaffold DE loop
GSER

SEQ ID NO: 37 - protein, 5 aa, synthetic construct
  REGION 1..5: note = Tencon27 scaffold E strand
SYDLT

SEQ ID NO: 38 - protein, 5 aa, synthetic construct
  REGION 1..5: note = Tencon27 scaffold EF loop
GLKPG

SEQ ID NO: 39 - protein, 10 aa, synthetic construct
  REGION 1..10: note = Tencon27 scaffold F strand
TEYTVSIYGV

SEQ ID NO: 40 - protein, 7 aa, synthetic construct
  REGION 1..7: note = Tencon27 scaffold FG loop
KGGHRSN

SEQ ID NO: 41 - protein, 8 aa, synthetic construct
  REGION 1..8: note = Tencon27 scaffold G strand
PLSAIFTT

SEQ ID NO: 42 - protein, 15 aa, synthetic construct
  REGION 1..15: note = Tencon27 scaffold C strand and CD loop
DSFLIQYQESEKVGE

SEQ ID NO: 43 - protein, 17 aa, synthetic construct
  REGION 1..17: note = Tencon27 scaffold F strand and FG loop
TEYTVSIYGVKGGHRSN

SEQ ID NO: 44 - protein, 28 aa, synthetic construct
  REGION 1..28: note = Tencon27 scaffold A strand, AB loop, B strand and BC loop
LPAPKNLVVSRVTEDSARLSWTAPDAAF

SEQ ID NO: 45 - protein, 9 aa, synthetic construct
  REGION 1..9: note = TCL14 library C strand
  SITE 4: note = misc_feature - Xaa can be any naturally occurring amino acid
  SITE 6: note = misc_feature - Xaa can be any naturally occurring amino acid
  SITE 8: note = misc_feature - Xaa can be any naturally occurring amino acid
DSFXIXYXE

SEQ ID NO: 46 - protein, 10 aa, synthetic construct
  REGION 1..10: note = TCL14 library F strand
  SITE 4: note = misc_feature - Xaa can be any naturally occurring amino acid
  SITE 6: note = misc_feature - Xaa can be any naturally occurring amino acid
  SITE 8: note = misc_feature - Xaa can be any naturally occurring amino acid
TEYXVXIXGV

SEQ ID NO: 47 - protein, 15 aa, synthetic construct
  REGION 1..15: note = TCL14 library C strand and CD loop
  SITE 4: note = misc_feature - Xaa can be any naturally occurring amino acid
  SITE 6: note = misc_feature - Xaa can be any naturally occurring amino acid
  SITE 8: note = misc_feature - Xaa can be any naturally occurring amino acid
  REGION 10..13: note = misc_feature - Xaa can be any naturally occurring amino acid
DSFXIXYXEXXXXGE

SEQ ID NO: 48 - protein, 17 aa, synthetic construct
  REGION 1..17: note = TCL14 library F strand and FG loop
  SITE 4: note = misc_feature - Xaa can be any naturally occurring amino acid
  SITE 6: note = misc_feature - Xaa can be any naturally occurring amino acid
  SITE 8: note = misc_feature - Xaa can be any naturally occurring amino acid
  REGION 14..15: note = misc_feature - Xaa can be any naturally occurring amino acid
  SITE 17: note = misc_feature - Xaa can be any naturally occurring amino acid
TEYXVXIXGVKGGXXSX

SEQ ID NO: 49 - protein, 28 aa, synthetic construct
  REGION 1..28: note = TCL15 library A strand, AB loop, B strand and BC loop
  SITE 6: note = misc_feature - Xaa can be any naturally occurring amino acid
  SITE 8: note = misc_feature - Xaa can be any naturally occurring amino acid
  REGION 10..11: note = misc_feature - Xaa can be any naturally occurring amino acid
  REGION 13..16: note = misc_feature - Xaa can be any naturally occurring amino acid
  SITE 18: note = misc_feature - Xaa can be any naturally occurring amino acid
  SITE 20: note = misc_feature - Xaa can be any naturally occurring amino acid
  SITE 22: note = misc_feature - Xaa can be any naturally occurring amino acid
LPAPKXLXVXXVXXXXAXLXWXAPDAAF

SEQ ID NO: 50 - skipped

SEQ ID NO: 51 - DNA, 126 bp, synthetic construct
  misc_feature 1..126: note = primer
  misc_feature 19..20: note = n is a, c, g, or t
  misc_feature 21: note = s is g or c
  misc_feature 25..26: note = n is a, c, g, or t
  misc_feature 27: note = s is g or c
  misc_feature 31..32: note = n is a, c, g, or t
  misc_feature 33: note = s is g or c
  misc_feature 37..38: note = n is a, c, g, or t
  misc_feature 39: note = s is g or c
  misc_feature 40..41: note = n is a, c, g, or t
  misc_feature 42: note = s is g or c
  misc_feature 43..44: note = n is a, c, g, or t
  misc_feature 45: note = s is g or c
  misc_feature 46..47: note = n is a, c, g, or t
  misc_feature 48: note = s is g or c
  source 1..126: mol_type = other DNA
gcggcgttcgactctttcnnsatcnnstacnnsgaannsnnsnnsnnsggtgaagcgatcggtctgaccgttccgggttctgaacgttcttacgacctgaccggtctgaaaccgggtaccgaatac

SEQ ID NO: 52 - DNA, 102 bp, synthetic construct
  misc_feature 1..102: note = primer
  misc_feature 25: note = s is c or g
  misc_feature 26..27: note = n is a, c, g, or t
  misc_feature 31: note = s is c or g
  misc_feature 32..33: note = n is a, c, g, or t
  misc_feature 34: note = s is c or g
  misc_feature 35..36: note = n is a, c, g, or t
  misc_feature 52: note = s is c or g
  misc_feature 53..54: note = n is a, c, g, or t
  misc_feature 58: note = s is c or g
  misc_feature 59..60: note = n is a, c, g, or t
  misc_feature 64: note = s is c or g
  misc_feature 65..66: note = n is a, c, g, or t
  source 1..102: mol_type = other DNA
ggtggtgaagatcgcagacagcggsnnagasnnsnnaccacctttaacaccsnngatsnnaacsnngtattcggtacccggtttcagaccggtcaggtcgta

SEQ ID NO: 53 - DNA, 27 bp, synthetic construct
  misc_feature 1..27: note = primer
  source 1..27: mol_type = other DNA
gaacgcggctacaattaatacataacc

SEQ ID NO: 54 - DNA, 22 bp, synthetic construct
  misc_feature 1..22: note = primer
  source 1..22: mol_type = other DNA
catgattacgccaagctcagaa

SEQ ID NO: 55 - DNA, 37 bp, synthetic construct
  misc_feature 1..37: note = primer
  source 1..37: mol_type = other DNA
aagaaggagaaccggtatgctgccggcgccgaaaaac

SEQ ID NO: 56 - DNA, 65 bp, synthetic construct
  misc_feature 1..65: note = primer
  source 1..65: mol_type = other DNA
gagccgccgccaccggtttaatggtgatggtgatggtgaccaccggtggtgaagatcgcagacag

SEQ ID NO: 57 - protein, 2201 aa, homo sapiens
MGAMTQLLAGVFLAFLALATEGGVLKKVIRHKRQSGVNATLPEENQPVVFNHVYNIKLPVGSQCSVDLESASGEKDLAPPSEPSESFQEHTVDGENQIVFTHRINIPRRACGCAAAPDVKELLSRLEELENLVSSLREQCTAGAGCCLQPATGRLDTRPFCSGRGNFSTEGCGCVCEPGWKGPNCSEPECPGNCHLRGRCIDGQCICDDGFTGEDCSQLACPSDCNDQGKCVNGVCICFEGYAGADCSREICPVPCSEEHGTCVDGLCVCHDGFAGDDCNKPLCLNNCYNRGRCVENECVCDEGFTGEDCSELICPNDCFDRGRCINGTCYCEEGFTGEDCGKPTCPHACHTQGRCEEGQCVCDEGFAGVDCSEKRCPADCHNRGRCVDGRCECDDGFTGADCGELKCPNGCSGHGRCVNGQCVCDEGYTGEDCSQLRCPNDCHSRGRCVEGKCVCEQGFKGYDCSDMSCPNDCHQHGRCVNGMCVCDDGYTGEDCRDRQCPRDCSNRGLCVDGQCVCEDGFTGPDCAELSCPNDCHGQGRCVNGQCVCHEGFMGKDCKEQRCPSDCHGQGRCVDGQCICHEGFTGLDCGQHSCPSDCNNLGQCVSGRCICNEGYSGEDCSEVSPPKDLVVTEVTEETVNLAWDNEMRVTEYLVVYTPTHEGGLEMQFRVPGDQTSTIIQELEPGVEYFIRVFAILENKKSIPVSARVATYLPAPEGLKFKSIKETSVEVEWDPLDIAFETWEIIFRNMNKEDEGEITKSLRRPETSYRQTGLAPGQEYEISLHIVKNNTRGPGLKRVTTTRLDAPSQIEVKDVTDTTALITWFKPLAEIDGIELTYGIKDVPGDRTTIDLTEDENQYSIGNLKPDTEYEVSLISRRGDMSSNPAKETFTTGLDAPRNLRRVSQTDNSITLEWRNGKAAIDSYRIKYAPISGGDHAEVDVPKSQQATTKTTLTGLRPGTEYGIGVSAVKEDKESNPATINAATELDTPKDLQVSETAETSLTLLWKTPLAKFDRYRLNYSLPTGQWVGVQLPRNTTSYVLRGLEPGQEYNVLLTAEKGRHKSKPARVKASTEQAPELENLTVTEVGWDGLRLNWTAADQAYEHFIIQVQEANKVEAARNLTVPGSLRAVDIPGLKAATPYTVSIYGVIQGYRTPVLSAEASTGETPNLGEVVVAEVGWDALKLNWTAPEGAYEYFFIQVQEADTVEAAQNLTVPGGLRSTDLPGLKAATHYTITIRGVTQDFSTTPLSVEVLTEEVPDMGNLTVTEVSWDALRLNWTTPDGTYDQFTIQVQEADQVEEAHNLTVPGSLRSMEIPGLRAGTPYTVTLHGEVRGHSTRPLAVEVVTEDLPQLGDLAVSEVGWDGLRLNWTAADNAYEHFVIQVQEVNKVEAAQNLTLPGSLRAVDIPGLEAATPYRVSIYGVIRGYRTPVLSAEASTAKEPEIGNLNVSDITPESFNLSWMATDGIFETFTIEIIDSNRLLETVEYNISGAERTAHISGLPPSTDFIVYLSGLAPSIRTKTISATATTEALPLLENLTISDINPYGFTVSWMASENAFDSFLVTVVDSGKLLDPQEFTLSGTQRKLELRGLITGIGYEVMVSGFTQGHQTKPLRAEIVTEAEPEVDNLLVSDATPDGFRLSWTADEGVFDNFVLKIRDTKKQSEPLEITLLAPERTRDITGLREATEYEIELYGISKGRRSQTVSAIATTAMGSPKEVIFSDITENSATVSWRAPTAQVESFRITYVPITGGTPSMVTVDGTKTQTRLVKLIPGVEYLVSIIAMKGFEESEPVSGSFTTALDGPSGLVTANITDSEALARWQPAIATVDSYVISYTGEKVPEITRTVSGNTVEYALTDLEPATEYTLRIFAEKGPQKSSTITAKFTTDLDSPRDLTATEVQSETALLTWRPPRASVTGYLLVYESVDGTVKEVIVGPDTTSYSLADLSPSTHYTAKIQALNGPLRSNMIQTIFTTIGLLYPFPKDCSQAMLNGDTTSGLYTIYLNGDKAEALEVFCDMTSDGGGWIVFLRRKNGRENFYQNWKAYAAGFGDRREEFWLGLDNLNKITAQGQYELRVDLRDHGETAFAVYDKFSVGDAKTRYKLKVEGYSGTAGDSMAYHNGRSFSTFDKDTDSAITNCALSYKGAFWYRNCHRVNLMGRYGDNNHSQGVNWFHWKGHEHSIQFAEMKLRPSNFRNLEGRRKRA

SEQ ID NO: 58 - protein, 89 aa, synthetic construct
  REGION 1..89: note = FN3 scaffold based on consensuns fibronecting FN3 domains
LDAPTDLQVTNVTDTSITVSWTPPSATITGYRITYTPSNGPGEPKELTVPPSSTSVTITGLTPGVEYVVSLYALKDNQESPPLVGTQTT

SEQ ID NO: 59 - DNA, 267 bp, synthetic construct
  misc_feature 1..267: note = cDNA encoding tencon scaffold
  source 1..267: mol_type = other DNA
ctgccggcgccgaaaaacctggttgtttctgaagttaccgaagactctctgcgtctgtcttggaccgcgccggacgcggcgttcgactctttcctgatccagtaccaggaatctgaaaaagttggtgaagcgatcaacctgaccgttccgggttctgaacgttcttacgacctgaccggtctgaaaccgggtaccgaatacaccgtttctatctacggtgttaaaggtggtcaccgttctaacccgctgtctgcggaattcaccacc

SEQ ID NO: 60 - protein, 7 aa, synthetic construct
  REGION 1..7: note = linker
TSGGGGS

SEQ ID NO: 61 - protein, 89 aa, synthetic construct
  REGION 1..89: note = TCL15 library on tencon27 having randomized A-AB-B-BC-E surface
  SITE 6: note = misc_feature - Xaa can be any naturally occurring amino acid
  SITE 8: note = misc_feature - Xaa can be any naturally occurring amino acid
  REGION 10..11: note = misc_feature - Xaa can be any naturally occurring amino acid
  REGION 13..16: note = misc_feature - Xaa can be any naturally occurring amino acid
  SITE 18: note = misc_feature - Xaa can be any naturally occurring amino acid
  SITE 20: note = misc_feature - Xaa can be any naturally occurring amino acid
  SITE 22: note = misc_feature - Xaa can be any naturally occurring amino acid
  SITE 55: note = misc_feature - Xaa can be any naturally occurring amino acid
  SITE 57: note = misc_feature - Xaa can be any naturally occurring amino acid
LPAPKXLXVXXVXXXXAXLXWXAPDAAFDSFLIQYQESEKVGEAIVLTVPGSERXYXLTGLKPGTEYTVSIYGVKGGHRSNPLSAIFTT

SEQ ID NO: 62 - protein, 89 aa, synthetic construct
  REGION 1..89: note = Fibcon library with randomized C-CD-F-FG surface
  SITE 32: note = misc_feature - Xaa can be any naturally occurring amino acid
  SITE 34: note = misc_feature - Xaa can be any naturally occurring amino acid
  SITE 36: note = misc_feature - Xaa can be any naturally occurring amino acid
  REGION 38..41: note = misc_feature - Xaa can be any naturally occurring amino acid
  SITE 68: note = misc_feature - Xaa can be any naturally occurring amino acid
  SITE 70: note = misc_feature - Xaa can be any naturally occurring amino acid
  SITE 72: note = misc_feature - Xaa can be any naturally occurring amino acid
  REGION 78..79: note = misc_feature - Xaa can be any naturally occurring amino acid
  SITE 81: note = misc_feature - Xaa can be any naturally occurring amino acid
LDAPTDLQVTNVTDTSITVSWTPPSATITGYXIXYXPXXXXGEPKELTVPPSSTSVTITGLTPGVEYXVXLXALKDNXXSXPLVGTQTT

SEQ ID NO: 63 - protein, 9 aa, synthetic construct
  REGION 1..9: note = C strand sequence of scaffold TP1KR9P61-A2
DSFAIEYFE

SEQ ID NO: 64 - protein, 9 aa, synthetic construct
  REGION 1..9: note = C strand sequence of clone TP1KR9P62-A2
DSFAIEYSE

SEQ ID NO: 65 - protein, 9 aa, synthetic construct
  REGION 1..9: note = C strand sequence of clone TP1KR9P62-D4
DSFGIIYFE

SEQ ID NO: 66 - protein, 9 aa, synthetic construct
  REGION 1..9: note = C strand sequence of clone TP1KR9P62-E3
DSFGIEYFE

SEQ ID NO: 67 - protein, 6 aa, synthetic construct
  REGION 1..6: note = CD loop of TP1KR9P61-A2
DWWSGE

SEQ ID NO: 68 - protein, 6 aa, synthetic construct
  REGION 1..6: note = CD loop of TP1KR9P62-A2
DYWLGE

SEQ ID NO: 69 - protein, 6 aa, synthetic construct
  REGION 1..6: note = CD loop of TP1KR9P62-D4
DWWAGE

SEQ ID NO: 70 - protein, 6 aa, synthetic construct
  REGION 1..6: note = CD loop of TP1KR9P62-E3
DYWTGE

SEQ ID NO: 71 - protein, 10 aa, synthetic construct
  REGION 1..10: note = F strand of TP1KR9P61-A2
TEYAVSIRGV

SEQ ID NO: 72 - protein, 10 aa, synthetic construct
  REGION 1..10: note = F strand of TP1KR9P61-A7
TEYSVSIRGV

SEQ ID NO: 73 - protein, 10 aa, synthetic construct
  REGION 1..10: note = TP1KR9P62-A2
TEYGVSIRGV

SEQ ID NO: 74 - protein, 10 aa, synthetic construct
  REGION 1..10: note = F strand of TP1KR9P62-C3
TEYSVTIRGV

SEQ ID NO: 75 - protein, 7 aa, synthetic construct
  REGION 1..7: note = FG loop of TP1KR9P61-A2
KGGMPSA

SEQ ID NO: 76 - protein, 7 aa, synthetic construct
  REGION 1..7: note = FG loop of TP1KR9P61-A7
KGGYPSS

SEQ ID NO: 77 - protein, 7 aa, synthetic construct
  REGION 1..7: note = FG loop of TP1KR9P61-E2
KGGMPSP

SEQ ID NO: 78 - protein, 7 aa, synthetic construct
  REGION 1..7: note = FG loop of TP1KR9P61-G4
KGGYPSA

SEQ ID NO: 79 - protein, 7 aa, synthetic construct
  REGION 1..7: note = FG loop of TP1KR9P62-A2
KGGYPSP

SEQ ID NO: 80 - protein, 7 aa, synthetic construct
  REGION 1..7: note = FG loop of TP1KR9P62-C3
KGGPPSS

SEQ ID NO: 81 - protein, 7 aa, synthetic construct
  REGION 1..7: note = FG loop of TP1KR9P62-C6
KGGYPSS

SEQ ID NO: 82 - protein, 7 aa, synthetic construct
  REGION 1..7: note = FG loop of TP1KR9P62-D4
KGGPPSR

SEQ ID NO: 83 - protein, 7 aa, synthetic construct
  REGION 1..7: note = FG loop of TP1KR9P62-D8
KGGLASP

SEQ ID NO: 84 - protein, 7 aa, synthetic construct
  REGION 1..7: note = FG loop of TP1KR9P62-H10
KGGHPSV

SEQ ID NO: 85 - protein, 90 aa, synthetic construct
  REGION 1..90: note = mIL-17A binding scaffold TP1KR9P61-A2
MLPAPKNLVVSRVTEDSARLSWTAPDAAFDSFAIEYFEDWWSGEAIVLTVPGSERSYDLTGLKPGTEYAVSIRGVKGGMPSAPLSAIFTT

SEQ ID NO: 86 - protein, 90 aa, synthetic construct
  REGION 1..90: note = mIL-17A binding scaffold TP1KR9P61-A7
MLPAPKNLVVSRVTEDSARLSWTAPDAAFDSFAIEYFEDWWSGEAIVLTVPGSERSYDLTGLKPGTEYSVSIRGVKGGYPSSPLSAIFTT

SEQ ID NO: 87 - protein, 90 aa, synthetic construct
  REGION 1..90: note = mIL-17A binding scaffold TP1KR9P61-E2
MLPAPKNLVVSRVTEDSARLSWTAPDAAFDSFAIEYFEDWWSGEAIVLTVPGSERSYDLTGLKPGTEYAVSIRGVKGGMPSPPLSAIFTT

SEQ ID NO: 88 - protein, 90 aa, synthetic construct
  REGION 1..90: note = mIL-17A binding scaffold TP1KR9P61-G4
MLPAPKNLVVSRVTEDSARLSWTAPDAAFDSFAIEYFEDWWSGEAIVLTVPGSERSYDLTGLKPGTEYAVSIRGVKGGYPSAPLSAIFTT

SEQ ID NO: 89 - protein, 90 aa, synthetic construct
  REGION 1..90: note = mIL-17A binding scaffold TP1KR9P62-A2
MLPALKNLVVSRVTEDSAHLSWTAPDAAFDSFAIEYSEDYWLGEAIVLTVPGSERSYDLTGLKPGTEYGVSIRGVKGGYPSPPLSAIFTT

SEQ ID NO: 90 - protein, 90 aa, synthetic construct
  REGION 1..90: note = mIL-17A binding scaffold TP1KR9P62-C3
MLPAPKNLVVSRVTEDSARLSWTAPDAAFDSFAIEYFEDWWSGEAIVLTVPGSERSYDLTGLKPGTEYSVTIRGVKGGPPSSPLSAIFTT

SEQ ID NO: 91 - protein, 90 aa, synthetic construct
  REGION 1..90: note = mIL-17A binding scaffold TP1KR9P62-C6
MLPAPKNLVVSRVTEDSARLSWTAPDAAFDSFAIEYFEDWWSGEAIVLTVPGSERSCDLTGLKPGTEYSVTIRGVKGGYPSSPLSAIFTT

SEQ ID NO: 92 - protein, 89 aa, synthetic construct
  REGION 1..89: note = mIL-17A binding scaffold TP1KR9P62-D3
MLPAPKNLVVSRVTEDSARLSWTAPDAAFDSFAIEYFEDWWSGEAIVLTVPGSERSYDLTLKPGTEYSVSIRGVKGGYPSSPLSAIFTT

SEQ ID NO: 93 - protein, 90 aa, synthetic construct
  REGION 1..90: note = mIL-17A binding scaffold TP1KR9P62-D4
MLPAPKNLVVSRVTEDSARLSWTAPDAAFDSFGIIYFEDWWAGEAIVLTVPGSERSYDLTGLKPGTEYGVSIRGVKGGPPSRPLSAIFTT

SEQ ID NO: 94 - protein, 90 aa, synthetic construct
  REGION 1..90: note = mIL-17A binding scaffold TP1KR9P62-D8
MLPAPKNLVVSRVTEDSARLSWTAPDAAFDSFAIEYFEDWWSGEAIVLTVPGSERSYDLTGLKPGTEYGVSIRGVKGGLASPPLSAIFTT

SEQ ID NO: 95 - protein, 90 aa, synthetic construct
  REGION 1..90: note = mIL-17A binding scaffold TP1KR9P62-E3
MLPAPKNLVVSRVTEDSARLSWTAPDAAFDSFGIEYFEDYWTGEAIVLTVPGSERSYDLTGLKPGTEYAVSIRGVKGGYPSAPLSAIFTT

SEQ ID NO: 96 - protein, 90 aa, synthetic construct
  REGION 1..90: note = mIL-17A binding scaffold TP1KR9P62-H10
MLPAPKNLVVSRVTEDSARLSWTAPDAAFDSFAIEYFEDWWSGEAIVLTVPGSERSYDLTGLKPGTEYSVSIRGVKGGHPSVPLSAIFTT

SEQ ID NO: 97 - protein, 94 aa, homo sapiens
VSDVPRDLEVVAATPTSLLISWDAPAVTVRYYRITYGETGGNSPVQEFTVPGSKSTATISGLKPGVDYTITVYAVTGRGDSPASSKPISINYRT

SEQ ID NO: 98 - protein, 94 aa, synthetic construct
  REGION 1..94: note = FN10 based scaffold library with randomized C-CD-F-FG surface
  SITE 33: note = misc_feature - Xaa can be any naturally occurring amino acid
  SITE 35: note = misc_feature - Xaa can be any naturally occurring amino acid
  SITE 37: note = misc_feature - Xaa can be any naturally occurring amino acid
  REGION 39..42: note = misc_feature - Xaa can be any naturally occurring amino acid
  SITE 69: note = misc_feature - Xaa can be any naturally occurring amino acid
  SITE 71: note = misc_feature - Xaa can be any naturally occurring amino acid
  SITE 73: note = misc_feature - Xaa can be any naturally occurring amino acid
  REGION 83..84: note = misc_feature - Xaa can be any naturally occurring amino acid
  SITE 86: note = misc_feature - Xaa can be any naturally occurring amino acid
VSDVPRDLEVVAATPTSLLISWDAPAVTVRYYXIXYXEXXXXSPVQEFTVPGSKSTATISGLKPGVDYXIXVXAVTGRGDSPXXSXPISINYRT

SEQ ID NO: 99 - protein, 88 aa, synthetic construct
  REGION 1..88: note = TN3 based scaffodl library with randomized C-CD-F-FG surface
  SITE 31: note = misc_feature - Xaa can be any naturally occurring amino acid
  SITE 33: note = misc_feature - Xaa can be any naturally occurring amino acid
  SITE 35: note = misc_feature - Xaa can be any naturally occurring amino acid
  REGION 37..40: note = misc_feature - Xaa can be any naturally occurring amino acid
  SITE 67: note = misc_feature - Xaa can be any naturally occurring amino acid
  SITE 69: note = misc_feature - Xaa can be any naturally occurring amino acid
  SITE 71: note = misc_feature - Xaa can be any naturally occurring amino acid
  REGION 77..78: note = misc_feature - Xaa can be any naturally occurring amino acid
  SITE 80: note = misc_feature - Xaa can be any naturally occurring amino acid
DAPSQIEVKDVTDTTALITWFKPLAEIDGIXLXYXIXXXXGDRTTIDLTEDENQYSIGNLKPDTEYXVXLXSRRGDXXSXPAKETFTT

SEQ ID NO: 100 - DNA, 270 bp, synthetic construct
  misc_feature 1..270: note = cDNA encoding tencon27
  source 1..270: mol_type = other DNA
atgctgccggcgccgaaaaacctggttgtttctcgtgttaccgaagactctgcgcgtctgtcttggaccgcgccggacgcggcgttcgactctttcctgatccagtaccaggaatctgaaaaagttggtgaagcgatcgttctgaccgttccgggttctgaacgttcttacgacctgaccggtctgaaaccgggtaccgaatacaccgtttctatctacggtgttaaaggtggtcaccgttctaacccgctgtctgcgatcttcaccacc

SEQ ID NO: 101 - DNA, 270 bp, synthetic construct
  misc_feature 1..270: note = cDNA encoding TCL14 library
  misc_feature 97..98: note = n is a, c, g, or t
  misc_feature 99: note = s is c or g
  misc_feature 103..104: note = n is a, c, g, or t
  misc_feature 105: note = s is c or g
  misc_feature 109..110: note = n is a, c, g, or t
  misc_feature 111: note = s is c or g
  misc_feature 115..116: note = n is a, c, g, or t
  misc_feature 117: note = s is c or g
  misc_feature 118..119: note = n is a, c, g, or t
  misc_feature 120: note = s is c or g
  misc_feature 121..122: note = n is a, c, g, or t
  misc_feature 123: note = s is c or g
  misc_feature 124..125: note = n is a, c, g, or t
  misc_feature 126: note = s is c or g
  misc_feature 205..206: note = n is a, c, g, or t
  misc_feature 207: note = s is c or g
  misc_feature 211..212: note = n is a, c, g, or t
  misc_feature 213: note = s is c or g
  misc_feature 217..218: note = n is a, c, g, or t
  misc_feature 219: note = s is c or g
  misc_feature 235..236: note = n is a, c, g, or t
  misc_feature 237: note = s is c or g
  misc_feature 238..239: note = n is a, c, g, or t
  misc_feature 240: note = s is c or g
  misc_feature 244..245: note = n is a, c, g, or t
  misc_feature 246: note = s is c or g
  source 1..270: mol_type = other DNA
atgctgccggcgccgaaaaacctggttgtttctcgtgttaccgaagactctgcgcgtctgtcttggaccgcgccggacgcggcgttcgactctttcnnsatcnnstacnnsgaannsnnsnnsnnsggtgaagcgatcgttctgaccgttccgggttctgaacgttcttacgacctgaccggtctgaaaccgggtaccgaatacnnsgttnnsatcnnsggtgttaaaggtggtnnsnnstctnnsccgctgtctgcgatcttcaccacc